European Patent Application EP 4 772 650 A1, published July 8, 2026. Title: 用于毛细管电泳分析的引物/探针组合物、检测方法及应用. Applicant: 宁波海尔施基因科技股份有限公司. Application WO. The sequence listing filed with the application follows.

SEQUENCE LISTING (61 sequences)

SEQ ID NO: 1 - DNA, 22 bp, synthetic construct
  source 1..22: mol_type = other DNA
gaagcatggtatgaatttcgtg

SEQ ID NO: 2 - DNA, 24 bp, synthetic construct
  source 1..24: mol_type = other DNA
ggaggaagtaaacactcagaaaga

SEQ ID NO: 3 - DNA, 20 bp, synthetic construct
  source 1..20: mol_type = other DNA
cttgaaccattgcagtcacc

SEQ ID NO: 4 - DNA, 24 bp, synthetic construct
  source 1..24: mol_type = other DNA
tcttctaaccgaggtcgaaacgta

SEQ ID NO: 5 - DNA, 24 bp, synthetic construct
  source 1..24: mol_type = other DNA
cgtacgaacactttatcaccacta

SEQ ID NO: 6 - DNA, 24 bp, synthetic construct
  source 1..24: mol_type = other DNA
caggcaagttaaggttagatagca

SEQ ID NO: 7 - DNA, 23 bp, synthetic construct
  source 1..23: mol_type = other DNA
agccacaacacttaaattcactc

SEQ ID NO: 8 - DNA, 20 bp, synthetic construct
  source 1..20: mol_type = other DNA
gacagaacccggtatttcag

SEQ ID NO: 9 - DNA, 25 bp, synthetic construct
  source 1..25: mol_type = other DNA
catatcttaatccgcaataccactc

SEQ ID NO: 10 - DNA, 22 bp, synthetic construct
  source 1..22: mol_type = other DNA
ctacttcagcaaatttgaccca

SEQ ID NO: 11 - DNA, 24 bp, synthetic construct
  source 1..24: mol_type = other DNA
ctcaccagaagttgtttgtatcac

SEQ ID NO: 12 - DNA, 21 bp, synthetic construct
  source 1..21: mol_type = other DNA
ttagggtgggaactctaacga

SEQ ID NO: 13 - DNA, 24 bp, synthetic construct
  source 1..24: mol_type = other DNA
tcagtagtagaccatgtgaattcc

SEQ ID NO: 14 - DNA, 24 bp, synthetic construct
  source 1..24: mol_type = other DNA
ttctccgttggcttagtaaatgtc

SEQ ID NO: 15 - DNA, 22 bp, synthetic construct
  source 1..22: mol_type = other DNA
ttgatctagaaattgccctcct

SEQ ID NO: 16 - DNA, 22 bp, synthetic construct
  source 1..22: mol_type = other DNA
ctacaagcgcgtgtatgatgag

SEQ ID NO: 17 - DNA, 20 bp, synthetic construct
  source 1..20: mol_type = other DNA
acctgcacaattacagccaa

SEQ ID NO: 18 - DNA, 26 bp, synthetic construct
  source 1..26: mol_type = other DNA
ccactctggtcatatgcattcaatct

SEQ ID NO: 19 - DNA, 25 bp, synthetic construct
  source 1..25: mol_type = other DNA
ctcgtcttgaaggaagtacaatcta

SEQ ID NO: 20 - DNA, 21 bp, synthetic construct
  source 1..21: mol_type = other DNA
gtcttgtctttagccattcca

SEQ ID NO: 21 - DNA, 22 bp, synthetic construct
  source 1..22: mol_type = other DNA
agccactaattgcattaccaag

SEQ ID NO: 22 - DNA, 22 bp, synthetic construct
  source 1..22: mol_type = other DNA
tgaagattaatgcggcttgtag

SEQ ID NO: 23 - DNA, 21 bp, synthetic construct
  source 1..21: mol_type = other DNA
gatgagctagtgtgcaaatgg

SEQ ID NO: 24 - DNA, 22 bp, synthetic construct
  source 1..22: mol_type = other DNA
agtttggcaattcatcctccac

SEQ ID NO: 25 - DNA, 25 bp, synthetic construct
  source 1..25: mol_type = other DNA
ctagcatcagttaacggattaatgg

SEQ ID NO: 26 - DNA, 22 bp, synthetic construct
  source 1..22: mol_type = other DNA
gcttaataggcaatgcattcca

SEQ ID NO: 27 - DNA, 22 bp, synthetic construct
  source 1..22: mol_type = other DNA
gtttaagagtcagcgcgcagta

SEQ ID NO: 28 - DNA, 19 bp, synthetic construct
  source 1..19: mol_type = other DNA
ccattactagcaattccga

SEQ ID NO: 29 - DNA, 24 bp, synthetic construct
  source 1..24: mol_type = other DNA
ctgtgaatatgggaggtttcatca

SEQ ID NO: 30 - DNA, 24 bp, synthetic construct
  source 1..24: mol_type = other DNA
ggaggtaagctctagtatgtaagg

SEQ ID NO: 31 - DNA, 22 bp, synthetic construct
  source 1..22: mol_type = other DNA
ccaattcggttcagtctaatcc

SEQ ID NO: 32 - DNA, 20 bp, synthetic construct
  source 1..20: mol_type = other DNA
catgtccttatgccgctttc

SEQ ID NO: 33 - DNA, 30 bp, synthetic construct
  source 1..30: mol_type = other DNA
atgcataacagcatcaacaccaacacgact

SEQ ID NO: 34 - DNA, 31 bp, synthetic construct
  source 1..31: mol_type = other DNA
taaatggaacattcctcaaacaccccaatgg

SEQ ID NO: 35 - DNA, 32 bp, synthetic construct
  source 1..32: mol_type = other DNA
acgtaaaatccagaatcagggtgatcctctaa

SEQ ID NO: 36 - DNA, 34 bp, synthetic construct
  source 1..34: mol_type = other DNA
tcaggccccctcaaagccgagatcgcacagagac

SEQ ID NO: 37 - DNA, 36 bp, synthetic construct
  source 1..36: mol_type = other DNA
atgttctaagcacgctaatctctatagagcatatgt

SEQ ID NO: 38 - DNA, 27 bp, synthetic construct
  source 1..27: mol_type = other DNA
ttagcagacaaattcccagttcttcac

SEQ ID NO: 39 - DNA, 35 bp, synthetic construct
  source 1..35: mol_type = other DNA
atcattgagacctaccataacccacctatcaggac

SEQ ID NO: 40 - DNA, 37 bp, synthetic construct
  source 1..37: mol_type = other DNA
ttcaataatgcgcacatcaggatcatagctgtccacc

SEQ ID NO: 41 - DNA, 25 bp, synthetic construct
  source 1..25: mol_type = other DNA
aaaagcgctgcatatgacccagtta

SEQ ID NO: 42 - DNA, 41 bp, synthetic construct
  source 1..41: mol_type = other DNA
tacattgcattcatcaatttgtagcacctgacgatcattag

SEQ ID NO: 43 - DNA, 40 bp, synthetic construct
  source 1..40: mol_type = other DNA
aagaccaacttcagcgcactctcgaggacgccgaggctct

SEQ ID NO: 44 - DNA, 50 bp, synthetic construct
  source 1..50: mol_type = other DNA
ctttgaggatttgctccatcttacgatattgctaccttctgtactggcca

SEQ ID NO: 45 - DNA, 43 bp, synthetic construct
  source 1..43: mol_type = other DNA
agaactacaaattatcactttgatactagccctattaatcgca

SEQ ID NO: 46 - DNA, 20 bp, synthetic construct
  source 1..20: mol_type = other DNA
caggtcctcgtcgccgtaca

SEQ ID NO: 47 - DNA, 42 bp, synthetic construct
  source 1..42: mol_type = other DNA
tcagctaatgacaactcgagccttactggcgatatggtccaa

SEQ ID NO: 48 - DNA, 37 bp, synthetic construct; identical to SEQ ID NO: 40
  source 1..37: mol_type = other DNA

SEQ ID NO: 49 - DNA, 43 bp, synthetic construct
  source 1..43: mol_type = other DNA
tacattgcattcatcaatttgtagcacctgacgatcagatctt

SEQ ID NO: 50 - DNA, 50 bp, synthetic construct
  source 1..50: mol_type = other DNA
taatagttatgtcatccctcttattaatcatcatcctagccctttcagac

SEQ ID NO: 51 - DNA, 41 bp, synthetic construct; identical to SEQ ID NO: 42
  source 1..41: mol_type = other DNA

SEQ ID NO: 52 - DNA, 31 bp, synthetic construct; identical to SEQ ID NO: 34
  source 1..31: mol_type = other DNA

SEQ ID NO: 53 - DNA, 42 bp, synthetic construct; identical to SEQ ID NO: 47
  source 1..42: mol_type = other DNA

SEQ ID NO: 54 - DNA, 31 bp, synthetic construct; identical to SEQ ID NO: 34
  source 1..31: mol_type = other DNA

SEQ ID NO: 55 - DNA, 31 bp, synthetic construct; identical to SEQ ID NO: 34
  source 1..31: mol_type = other DNA

SEQ ID NO: 56 - DNA, 37 bp, synthetic construct; identical to SEQ ID NO: 40
  source 1..37: mol_type = other DNA

SEQ ID NO: 57 - DNA, 42 bp, synthetic construct; identical to SEQ ID NO: 47
  source 1..42: mol_type = other DNA

SEQ ID NO: 58 - DNA, 49 bp, synthetic construct
  source 1..49: mol_type = other DNA
taatagttatgtcatccctcttattaatcatcatcctagccctaagtct

SEQ ID NO: 59 - DNA, 20 bp, synthetic construct
  source 1..20: mol_type = other DNA
ataagactcggcggttactc

SEQ ID NO: 60 - DNA, 40 bp, synthetic construct
  source 1..40: mol_type = other DNA
agtgtaagactcggcggtttggtacttcacactacacacg

SEQ ID NO: 61 - DNA, 70 bp, synthetic construct
  source 1..70: mol_type = other DNA
tccatcaggacggggaataactatctccaacgtacattggcactgatttagatggtgacgacctgtgccg